European Patent Application EP 4 378 458 A1, published June 5, 2024. Title: A Composition for Preventing or Treating Metabolic Disorders Comprising Benzylaminoethanol Devatives as Active Ingredients. Applicant: 연세대학교 산학협력단. The sequence listing filed with the application follows.

SEQUENCE LISTING (6 sequences)

SEQ ID NO: 1 - DNA, 20 bp, synthetic construct
  source 1..20: mol_type = other DNA
agggcgatcttgacaggaaa

SEQ ID NO: 2 - DNA, 20 bp, synthetic construct
  source 1..20: mol_type = other DNA
cgaaactggcacccttgaaa

SEQ ID NO: 3 - DNA, 20 bp, synthetic construct
  source 1..20: mol_type = other DNA
gtgactttgactacccggga

SEQ ID NO: 4 - DNA, 20 bp, synthetic construct
  source 1..20: mol_type = other DNA
ggggctcttgtttgatcacc

SEQ ID NO: 5 - DNA, 20 bp, synthetic construct
  source 1..20: mol_type = other DNA
tgggttctagccagcagagt

SEQ ID NO: 6 - DNA, 20 bp, synthetic construct
  source 1..20: mol_type = other DNA
accaccagagaccgttatgc